European Patent Application EP 4 644 416 A2, published November 5, 2025. Title: INTERLEUKIN 5 BINDING PROTEIN DOSAGE REGIMEN. Applicant: GlaxoSmithKline Intellectual Property Development Limited. The sequence listing filed with the application follows.

SEQUENCE LISTING (19 sequences)

SEQ ID NO: 1 - protein, 449 aa, synthetic construct
  REGION 1..449: note = Full length heavy chain
QVTLRESGPALVKPTQTLTLTCTVSGFSLTGSSVHWVRQPPGKGLEWLGVIWASGGTDYNSALMSRLSISKDTSRNQVVLTMTNMDPVDTATYYCARDPPSGLLRLDYWGRGTLVTVSSASTKGPSVFPLAPSSKSTSGGTAALGCLVKDYFPEPVTVSWNSGALTSGVHTFPAVLQSSGLYSLSSVVTVPSSSLGTQTYICNVNHKPSNTKVDKRVEPKSCDKTHTCPPCPAPELLGGPSVFLFPPKPKDTLYITREPEVTCVVVDVSHEDPEVKFNWYVDGVEVHNAKTKPREEQYNSTYRVVSVLTVLHQDWLNGKEYKCKVSNKALPAPIEKTISKAKGQPREPQVYTLPPSREEMTKNQVSLTCLVKGFYPSDIAVEWESNGQPENNYKTTPPVLDSDGSFFLYSKLTVDKSRWQQGNVFSCSVMHEALHNHYTQKSLSLSPGK

SEQ ID NO: 2 - protein, 220 aa, synthetic construct
  REGION 1..220: note = Full length light chain
DIVMTQSPDSLAVSLGERATINCKSSQSLLNSGNQKNYLAWYQQKPGQPPKLLIYGASTRESGVPDRFSGSGSGTDFTLTISSLQAEDVAVYYCQNVHSFPFTFGGGTKLEIKRTVAAPSVFIFPPSDEQLKSGTASVVCLLNNFYPREAKVQWKVDNALQSGNSQESVTEQDSKDSTYSLSSTLTLSKADYEKHKVYACEVTHQGLSSPVTKSFNRGEC

SEQ ID NO: 3 - protein, 119 aa, synthetic construct
  REGION 1..119: note = VH sequence
QVTLRESGPALVKPTQTLTLTCTVSGFSLTGSSVHWVRQPPGKGLEWLGVIWASGGTDYNSALMSRLSISKDTSRNQVVLTMTNMDPVDTATYYCARDPPSGLLRLDYWGRGTLVTVSS

SEQ ID NO: 4 - protein, 114 aa, synthetic construct
  REGION 1..114: note = VL sequence
DIVMTQSPDSLAVSLGERATINCKSSQSLLNSGNQKNYLAWYQQKPGQPPKLLIYGASTRESGVPDRFSGSGSGTDFTLTISSLQAEDVAVYYCQNVHSFPFTFGGGTKLEIKR

SEQ ID NO: 5 - protein, 5 aa, synthetic construct
  REGION 1..5: note = CDRH1
GSSVH

SEQ ID NO: 6 - protein, 16 aa, synthetic construct
  REGION 1..16: note = CDRH2
VIWASGGTDYNSALMS

SEQ ID NO: 7 - protein, 11 aa, synthetic construct
  REGION 1..11: note = CDRH3
DPPSGLLRLDY

SEQ ID NO: 8 - protein, 17 aa, synthetic construct
  REGION 1..17: note = CDRL1
KSSQSLLNSGNQKNYLA

SEQ ID NO: 9 - protein, 7 aa, synthetic construct
  REGION 1..7: note = CDRL2
GASTRES

SEQ ID NO: 10 - protein, 9 aa, synthetic construct
  REGION 1..9: note = CDRL3
QNVHSFPFT

SEQ ID NO: 11 - protein, 115 aa, Homo sapiens
IPTEIPTSALVKETLALLSTHRTLLIANETLRIPVPVHKNHQLCTEEIFQGIGTLESQTVQGGTVERLFKNLSLIKKYIDGQKKKCGEERRRVNQFLDYLQEFLGVMNTEWIIES

SEQ ID NO: 12 - protein, 400 aa, Homo sapiens
DLLPDEKISLLPPVNFTIKVTGLAQVLLQWKPNPDQEQRNVNLEYQVKINAPKEDDYETRITESKCVTILHKGFSASVRTILQNDHSLLASSWASAELHAPPGSPGTSIVNLTCTTNTTEDNYSRLRSYQVSLHCTWLVGTDAPEDTQYFLYYRYGSWTEECQEYSKDTLGRNIACWFPRTFILSKGRDWLAVLVNGSSKHSAIRPFDQLFALHAIDQINPPLNVTAEIEGTRLSIQWEKPVSAFPIHCFDYEVKIHNTRNGYLQIEKLMTNAFISIIDDLSKYDVQVRAAVSSMCREAGLWSEWSQPIYVGNDEHKPLREWFVIVIMATICFILLILSLICKICHLWIKLFPPIPAPKSNIKDLFVTTNYEKAGSSETEIEVICYIEKPGVETLEDSVF

SEQ ID NO: 13 - DNA, 1404 bp, synthetic construct
  misc_feature 1..1404: note = DNA encoding full length heavy chain with leader sequence
  source 1..1404: mol_type = other DNA
atgggctggtcctgcatcatcctgtttctggtggccaccgccaccggtgtgcacagccaggtgaccctgagggagagcggccccgccctggtgaagcccacacagaccctcactctgacctgcaccgtgagcggcttcagcctgaccggctctagcgtccactgggtgaggcagccccccggcaagggcctggagtggctgggcgtgatctgggcaagcggggggacggactacaactcggccctgatgagcaggctctccatcagcaaggacaccagccggaaccaggtggtgctgaccatgaccaacatggaccccgtggacaccgccacctattactgcgccagggaccctccctccggcctgctgaggctggactactggggcaggggaacactagtgaccgtgtccagcgccagcaccaagggccccagcgtgttccccctggcccccagcagcaagagcaccagcggcggcacagccgccctgggctgcctggtgaaggactacttccccgagcccgtgaccgtgtcctggaacagcggagccctgaccagcggcgtgcacaccttccccgccgtgctgcagagcagcggcctgtacagcctgagcagcgtggtgaccgtgcccagcagcagcctgggcacccagacctacatctgtaacgtgaaccacaagcccagcaacaccaaggtggacaagcgggtggagcccaagagctgtgacaagacccacacctgccccccctgccctgcccccgagctgctgggaggccccagcgtgttcctgttcccccccaagcctaaggacaccctgtacatcaccagagaacccgaggtgacctgtgtggtggtggatgtgagccacgaggaccctgaggtgaagttcaactggtacgtggacggcgtggaggtgcacaatgccaagaccaagcccagggaggagcagtacaacagcacctaccgggtggtgtccgtgctgaccgtgctgcaccaggattggctgaacggcaaggagtacaagtgtaaggtgtccaacaaggccctgcctgcccctatcgagaaaaccatcagcaaggccaagggccagcccagagagccccaggtgtacaccctgccccctagcagagaggagatgaccaagaaccaggtgtccctgacctgcctggtgaagggcttctaccccagcgacatcgccgtggagtgggagagcaacggccagcccgagaacaactacaagaccaccccccctgtgctggacagcgatggcagcttcttcctgtacagcaagctgaccgtggacaagagcagatggcagcagggcaacgtgttcagctgctccgtgatgcacgaggccctgcacaatcactacacccagaagagcctgagcctgtcccctggcaag

SEQ ID NO: 14 - DNA, 717 bp, synthetic construct
  misc_feature 1..717: note = DNA encoding full length light chain with leader sequence
  source 1..717: mol_type = other DNA
atgggctggtcctgcatcatcctgtttctggtggccaccgccaccggtgtgcacagcgacatcgtgatgacccagtctcccgattcactggccgtgagcctgggcgagagggccaccatcaactgcaagagcagccagagcctcctgaacagcggcaaccagaagaactacctggcctggtaccagcagaaacccggccagccccccaagctgctgatctatggcgcctccaccagggagagcggcgtgccagacaggtttagcggcagcggcagcggcaccgacttcaccctgacaatcagcagcctgcaggccgaggacgtggccgtgtactactgccagaacgtccacagcttccccttcaccttcggcgggggaaccaagctggagatcaagcgtacggtggccgcccccagcgtgttcatcttcccccccagcgatgagcagctgaagagcggcaccgccagcgtggtgtgtctgctgaacaacttctacccccgggaggccaaggtgcagtggaaggtggacaatgccctgcagagcggcaacagccaggagagcgtgaccgagcaggacagcaaggactccacctacagcctgagcagcaccctgaccctgagcaaggccgactacgagaagcacaaggtgtacgcctgtgaggtgacccaccagggcctgtccagccccgtgaccaagagcttcaaccggggcgagtgc

SEQ ID NO: 15 - DNA, 357 bp, synthetic construct
  misc_feature 1..357: note = DNA encoding heavy chain variable region
  source 1..357: mol_type = other DNA
caggtgaccctgagggagagcggccccgccctggtgaagcccacacagaccctcactctgacctgcaccgtgagcggcttcagcctgaccggctctagcgtccactgggtgaggcagccccccggcaagggcctggagtggctgggcgtgatctgggcaagcggggggacggactacaactcggccctgatgagcaggctctccatcagcaaggacaccagccggaaccaggtggtgctgaccatgaccaacatggaccccgtggacaccgccacctattactgcgccagggaccctccctccggcctgctgaggctggactactggggcaggggaacactagtgaccgtgtccagc

SEQ ID NO: 16 - DNA, 342 bp, synthetic construct
  misc_feature 1..342: note = DNA encoding light chain variable region
  source 1..342: mol_type = other DNA
gacatcgtgatgacccagtctcccgattcactggccgtgagcctgggcgagagggccaccatcaactgcaagagcagccagagcctcctgaacagcggcaaccagaagaactacctggcctggtaccagcagaaacccggccagccccccaagctgctgatctatggcgcctccaccagggagagcggcgtgccagacaggtttagcggcagcggcagcggcaccgacttcaccctgacaatcagcagcctgcaggccgaggacgtggccgtgtactactgccagaacgtccacagcttccccttcaccttcggcgggggaaccaagctggagatcaagcgt

SEQ ID NO: 17 - DNA, 1347 bp, synthetic construct
  misc_feature 1..1347: note = DNA encoding full length heavy chain
  source 1..1347: mol_type = other DNA
caggtgaccctgagggagagcggccccgccctggtgaagcccacacagaccctcactctgacctgcaccgtgagcggcttcagcctgaccggctctagcgtccactgggtgaggcagccccccggcaagggcctggagtggctgggcgtgatctgggcaagcggggggacggactacaactcggccctgatgagcaggctctccatcagcaaggacaccagccggaaccaggtggtgctgaccatgaccaacatggaccccgtggacaccgccacctattactgcgccagggaccctccctccggcctgctgaggctggactactggggcaggggaacactagtgaccgtgtccagcgccagcaccaagggccccagcgtgttccccctggcccccagcagcaagagcaccagcggcggcacagccgccctgggctgcctggtgaaggactacttccccgagcccgtgaccgtgtcctggaacagcggagccctgaccagcggcgtgcacaccttccccgccgtgctgcagagcagcggcctgtacagcctgagcagcgtggtgaccgtgcccagcagcagcctgggcacccagacctacatctgtaacgtgaaccacaagcccagcaacaccaaggtggacaagcgggtggagcccaagagctgtgacaagacccacacctgccccccctgccctgcccccgagctgctgggaggccccagcgtgttcctgttcccccccaagcctaaggacaccctgtacatcaccagagaacccgaggtgacctgtgtggtggtggatgtgagccacgaggaccctgaggtgaagttcaactggtacgtggacggcgtggaggtgcacaatgccaagaccaagcccagggaggagcagtacaacagcacctaccgggtggtgtccgtgctgaccgtgctgcaccaggattggctgaacggcaaggagtacaagtgtaaggtgtccaacaaggccctgcctgcccctatcgagaaaaccatcagcaaggccaagggccagcccagagagccccaggtgtacaccctgccccctagcagagaggagatgaccaagaaccaggtgtccctgacctgcctggtgaagggcttctaccccagcgacatcgccgtggagtgggagagcaacggccagcccgagaacaactacaagaccaccccccctgtgctggacagcgatggcagcttcttcctgtacagcaagctgaccgtggacaagagcagatggcagcagggcaacgtgttcagctgctccgtgatgcacgaggccctgcacaatcactacacccagaagagcctgagcctgtcccctggcaag

SEQ ID NO: 18 - DNA, 660 bp, synthetic construct
  misc_feature 1..660: note = DNA encoding full length light chain
  source 1..660: mol_type = other DNA
gacatcgtgatgacccagtctcccgattcactggccgtgagcctgggcgagagggccaccatcaactgcaagagcagccagagcctcctgaacagcggcaaccagaagaactacctggcctggtaccagcagaaacccggccagccccccaagctgctgatctatggcgcctccaccagggagagcggcgtgccagacaggtttagcggcagcggcagcggcaccgacttcaccctgacaatcagcagcctgcaggccgaggacgtggccgtgtactactgccagaacgtccacagcttccccttcaccttcggcgggggaaccaagctggagatcaagcgtacggtggccgcccccagcgtgttcatcttcccccccagcgatgagcagctgaagagcggcaccgccagcgtggtgtgtctgctgaacaacttctacccccgggaggccaaggtgcagtggaaggtggacaatgccctgcagagcggcaacagccaggagagcgtgaccgagcaggacagcaaggactccacctacagcctgagcagcaccctgaccctgagcaaggccgactacgagaagcacaaggtgtacgcctgtgaggtgacccaccagggcctgtccagccccgtgaccaagagcttcaaccggggcgagtgc

SEQ ID NO: 19 - protein, 11 aa, synthetic construct
  REGION 1..11: note = Heavy chain FR4 sequence
WGRGTLVTVSS